European Patent Specification EP 4 127 202 B1, published July 9, 2025. Title: METHODS AND COMPOSITIONS FOR THE PRODUCTION OF XYLITOL FROM XYLOSE UTILIZING DYNAMIC METABOLIC CONTROL. Applicant: DUKE UNIVERSITY. The sequence listing filed with the application follows.

SEQUENCE LISTING (31 sequences)

SEQ ID NO: 1 - DNA, 1487 bp, Artificial Sequence
  Synthetic
gatacgatggcactggcgctgaaaattgcagcgcgcatgattgaagatggcgagctggataaacgcatcgcgcagcgttattccggctggaatagcgaattgggccagcaaatcctgaaaggccaaatgtcactggcagatttagccaaatatgctcaggaacatcatttgtctccggtgcatcagagtggtcgccaggaacaactggaaaatctggtaaaccattatctgttcgacaaagcggccaacgatgaaaactattctgaaaactatgcggatgcgtcttaatgataaggaccgtgttgacaattaatcatcggcatagtatatcggcatagtataatacgacaaggtgaggaactaaaccatgagtattcaacatttccgtgtcgcccttattcccttttttgcggcattttgccttcctgtttttgctcacccagaaacgctggtgaaagtaaaagatgctgaagatcagttgggtgcacgagtgggttacatcgaactggatctcaacagcggtaagatccttgagagtttacgccccgaagaacgttttccaatgatgagcacttttaaagttctgctatgtggcgcggtattatcccgtattgacgccgggcaagagcaactcggtcgccgcatacactattctcagaatgacttggttgagtactcaccagtcacagaaaagcatctcacggatggcatgacagtaagagaattatgcagtgctgccataaccatgagtgataacactgcggccaacttacttctggcaacgatcggaggaccgaaggagctaaccgcttttttgcacaacatgggggatcatgtaactcgccttgatcgttgggaaccggagctgaatgaagccataccaaacgacgagcgtgacaccacgatgcctgtagcaatggcaacaacgttgcgcaaactattaactggcgaactacttactctagcttcccggcaacaattaatagactggatggaggcggataaagttgcaggatcacttctgcgctcggccctcccggctggctggtttattgctgataaatctggagccggtgagcgtgggtctcgcggtatcattgcagcactggggccagatggtaagccctcccgcatcgtagttatctacacgacggggagtcaggcaactatggatgaacgaaatagacagatcgctgagataggtgcctcactgattaagcattggtagtaagtagggataacagggtaatcggctaactgtgcagtccgttggcccggttatcggtagcgataccgggcatttttttaaggaacgatcgatatgtatatcgggatagatcttggcacctcgggcgtaaaagttattttgctcaacgagcagggtgaggtggttgctgcgcaaacggaaaagctgaccgtttcgcgcccgcatccactctggtcggaacaagacccggaacagtggtggcaggcaactgatcgcgcaa

SEQ ID NO: 2 - DNA, 970 bp, Artificial Sequence
  Synthetic
ctattgaagatgtgggtaactctgcggcattcctgtgctccgatctctctgccggtatctccggtgaagtggtccacgttgacggcggtttcagcattgctgcaatgaacgaactcgaactgaaagcggccaacgatgaaaactattctgaaaactatgcggatgcgtcttaataggaagttcctattctctagaaagtataggaacttccgaatccatgtgggagtttattcttgacacagatatttatgatataataactgagtaagcttaacataaggaggaaaaacatatgttacgcagcagcaacgatgttacgcagcagggcagtcgccctaaaacaaagttaggtggctcaagtatgggcatcattcgcacatgtaggctcggccctgaccaagtcaaatccatgcgggctgctcttgatcttttcggtcgtgagttcggagacgtagccacctactcccaacatcagccggactccgattacctcgggaacttgctccgtagtaagacattcatcgcgcttgctgccttcgaccaagaagcggttgttggcgctctcgcggcttacgttctgcccaagtttgagcagccgcgtagtgagatctatatctatgatctcgcagtctccggcgagcaccggaggcagggcattgccaccgcgctcatcaatctcctcaagcatgaggccaacgcgcttggtgcttatgtgatctacgtgcaagcagattacggtgacgatcccgcagtggctctctatacaaagttgggcatacgggaagaagtgatgcactttgatatcgacccaagtaccgccacctaagaagttcctattctctagaaagtataggaacttccgttctgttggtaaagatgggcggcgttctgccgcccgttatctctgttatacctttctgatatttgttatcgccgatccgtctttctccccttcccgccttgcgtcagg

SEQ ID NO: 3 - DNA, 869 bp, Artificial Sequence
  Synthetic
gtattccgtcttccatgttcaccgtcattttcgcaatggcacgtaccgttggctggatcgcccactggagcgaaatgcacagtgacggtatgaagattgcccgtccgcgtcagctgtatacaggatatgaaaaacgcgactttaaaagcgatatcaagcgtgcggccaacgatgaaaactattctgaaaactatgcggatgcgtcttaatagttgacaattaatcatcggcatagtatatcggcatagtataatacgactcactataggagggccatcatggccaagttgaccagtgccgttccggtgctcaccgcgcgcgacgtcgccggagcggtcgagttctggaccgaccggctcgggttctcccgggacttcgtggaggacgacttcgccggtgtggtccgggacgacgtgaccctgttcatcagcgcggtccaggaccaggtggtgccggacaacaccctggcctgggtgtgggtgcgcggcctggacgagctgtacgccgagtggtcggaggtcgtgtccacgaacttccgggacgcctccgggccggccatgaccgagatcggcgagcagccgtgggggcgggagttcgccctgcgcgacccggccggcaactgcgtgcactttgtggcagaggagcaggactgaggataagtaatggttgattgctaagttgtaaatattttaacccgccgttcatatggcgggttgatttttatatgcctaaacacaaaaaattgtaaaaataaaatccattaacagacctatatagatatttaaaaagaatagaacagctcaaattatcagcaacccaatactttcaattaaaaacttcatggtagtcgcatttataaccctatgaaa

SEQ ID NO: 4 - DNA, 852 bp, Artificial Sequence
  Synthetic
tctgggtattcactgctttggcgagcgcgctgccgaaattattcatatcggtcaggcgattatggaacagaaaggtggcggcaacactattgagtacttcgtcaacaccacctttaactacccgacgatggcggaagcctatcgggtagctgcgttaaacggtttaaaccgcctgtttgcggccaacgatgaaaactattctgaaaactatgcggatgcgtcttaatagttgacaattaatcatcggcatagtatatcggcatagtataatacgactcactataggagggccatcatgaagaccttcaacatctctcagcaggatctggagctggtggaggtcgccactgagaagatcaccatgctctatgaggacaacaagcaccatgtcggggcggccatcaggaccaagactggggagatcatctctgctgtccacattgaggcctacattggcagggtcactgtctgtgctgaagccattgccattgggtctgctgtgagcaacgggcagaaggactttgacaccattgtggctgtcaggcacccctactctgatgaggtggacagatccatcagggtggtcagcccctgtggcatgtgcagagagctcatctctgactatgctcctgactgctttgtgctcattgagatgaatggcaagctggtcaaaaccaccattgaggaactcatccccctcaagtacaccaggaactaaagtaaaactttatcgaaatggccatccattcttgcgcggatggcctctgccagctgctcatagcggctgcgcagcggtgagccaggacgataaaccaggccaatagtgcggcgtggttccggcttaatgcacgg

SEQ ID NO: 5 - DNA, 898 bp, Artificial Sequence
  Synthetic
gaagtggaagaagcctggaaatgggtagactccattactgaggcgtgggcgatggacaatgatgcgccgaaaccgtatcaggccggaacctggggacccgttgcctcggtggcgatgattacccgtgatggtcgttcctggaatgagtttgaggcggccaacgatgaaaactattctgaaaactatgcggatgcgtcttaatagttgacaattaatcatcggcatagtatatcggcatagtataatacgactcactataggagggccatcatgaagaccttcaacatctctcagcaggatctggagctggtggaggtcgccactgagaagatcaccatgctctatgaggacaacaagcaccatgtcggggcggccatcaggaccaagactggggagatcatctctgctgtccacattgaggcctacattggcagggtcactgtctgtgctgaagccattgccattgggtctgctgtgagcaacgggcagaaggactttgacaccattgtggctgtcaggcacccctactctgatgaggtggacagatccatcagggtggtcagcccctgtggcatgtgcagagagctcatctctgactatgctcctgactgctttgtgctcattgagatgaatggcaagctggtcaaaaccaccattgaggaactcatccccctcaagtacaccaggaactaaagtaatatctgcgcttatcctttatggttattttaccggtaacatgatcttgcgcagattgtagaacaatttttacactttcaggcctcgtgcggattcacccacgaggctttttttattacactgactgaaacgtttttgccctatgagctccggttacaggcgtttcagtcataaatcctctgaatgaaacgcgttgtgaatc

SEQ ID NO: 6 - DNA, 93 bp, Artificial Sequence
  Synthetic
tcgagttccccgcgccagcggggataaaccgaaaagcatataatgcgtaaaagttatgaagttcgagttccccgcgccagcggggataaaccg

SEQ ID NO: 7 - DNA, 28 bp, Artificial Sequence
  Synthetic
ccggatgagcattcatcaggcgggcaag

SEQ ID NO: 8 - DNA, 47 bp, Artificial Sequence
  Synthetic
cggtttatccccgctggcgcggggaactcgaacttcataacttttac

SEQ ID NO: 9 - DNA, 63 bp, Artificial Sequence
  Synthetic
tattgaccaattcattcgggacagttattagttcgagttccccgcgccagcggggataaaccg

SEQ ID NO: 10 - DNA, 28 bp, Artificial Sequence
  Synthetic
ccggatgagcattcatcaggcgggcaag

SEQ ID NO: 11 - DNA, 44 bp, Artificial Sequence
  Synthetic
cggtttatccccgctggcgcggggaactcgaactaataactgtc

SEQ ID NO: 12 - DNA, 61 bp, Artificial Sequence
  Synthetic
ttaccattctgttgcttttatgtataagaatcgagttccccgcgccagcggggataaaccg

SEQ ID NO: 13 - DNA, 28 bp, Artificial Sequence
  Synthetic
ccggatgagcattcatcaggcgggcaag

SEQ ID NO: 14 - DNA, 48 bp, Artificial Sequence
  Synthetic
cggtttatccccgctggcgcggggaactcgattcttatacataaaagc

SEQ ID NO: 15 - DNA, 61 bp, Artificial Sequence
  Synthetic
ctcgtaaaagcagtacagtgcaccgtaagatcgagttccccgcgccagcggggataaaccg

SEQ ID NO: 16 - DNA, 28 bp, Artificial Sequence
  Synthetic
ccggatgagcattcatcaggcgggcaag

SEQ ID NO: 17 - DNA, 49 bp, Artificial Sequence
  Synthetic
cggtttatccccgctggcgcggggaactcgatcttacggtgcactgtac

SEQ ID NO: 18 - DNA, 61 bp, Artificial Sequence
  Synthetic
ggagtgcccaatattacgacatcatccatctcgagttccccgcgccagcggggataaaccg

SEQ ID NO: 19 - DNA, 34 bp, Artificial Sequence
  Synthetic
ccagcggggataaaccgggagtgcccaatattac

SEQ ID NO: 20 - DNA, 28 bp, Artificial Sequence
  Synthetic
cttgcccgcctgatgaatgctcatccgg

SEQ ID NO: 21 - DNA, 1655 bp, Artificial Sequence
  Synthetic
aaagacttccgcaaaatgctggctcattgcgaagccgttaccccgattcgccgtaccgttactattgaagatgtgggtaactctgcggcattcctgtgctccgatctctctgccggtatctccggtgaagtggtccacgttgacggcggtttcagcattgctgcaatgaacgaactcgaactgaaagggggttcaggcgggtcgggtggcgtgagcaagggcgaggagctgttcaccggggtggtgcccatcctggtcgagctggacggcgacgtaaacggccacaagttcagcgtgcgcggcgagggcgagggcgatgccaccaacggcaagctgaccctgaagttcatctgcaccaccggcaagctgcccgtgccctggcccaccctcgtgaccaccctgacctacggcgtgcagtgcttcagccgctaccccgaccacatgaagcgccacgacttcttcaagtccgccatgcccgaaggctacgtccaggagcgcaccatcagcttcaaggacgacggcacctacaagacccgcgccgaggtgaagttcgagggcgacaccctggtgaaccgcatcgagctgaagggcatcgacttcaaggaggacggcaacatcctggggcacaagctggagtacaacttcaacagccacaacgtctatatcaccgccgacaagcagaagaacggcatcaaggccaacttcaagatccgccacaacgtggaggacggcagcgtgcagctcgccgaccactaccagcagaacacccccatcggcgacggccccgtgctgctgcccgacaaccactacctgagcacccagtccgtgctgagcaaagaccccaacgagaagcgcgatcacatggtcctgctggagttcgtgaccgccgccgggatcactcacggcatggacgagctgtacaagtaatgacgaatccatgtgggagtttattcttgacacagatatttatgatataataactgagtaagcttaacataaggaggaaaaacatatgttgcgtagctctaacgatgtgacgcaacaaggttcgcgtccaaagacaaaattgggaggcagtagcatggggatcattcgcacttgtcgcctggggccagaccaggtgaagtcaatgcgtgcggctctggacttattcgggcgcgaatttggagatgtagccacttactcacagcaccaaccggacagtgattacttggggaatttacttcgcagtaaaacttttatcgctttggccgctttcgaccaggaggctgtagtaggtgcgttggcagcctatgttcttcctaaattcgagcaaccgcgtagcgaaatttacatctatgatcttgcagtctccggcgaacatcgccgtcaggggatcgccacagctttaatcaaccttttgaagcatgaggctaatgcacttggagcgtacgtgatttatgtgcaggctgactacggtgatgatcctgcagtcgctctgtacaccaaactgggtatccgcgaggaggtcatgcactttgatattgacccgtcgacggctacctaagttctgttggtaaagatgggcggcgttctgccgcccgttatctctgttatacctttctgatatttgttatcgccgatccgtctttctccccttcccgccttgcgtcagg

SEQ ID NO: 22 - DNA, 1730 bp, Artificial Sequence
  Synthetic
aaagacttccgcaaaatgctggctcattgcgaagccgttaccccgattcgccgtaccgttactattgaagatgtgggtaactctgcggcattcctgtgctccgatctctctgccggtatctccggtgaagtggtccacgttgacggcggtttcagcattgctgcaatgaacgaactcgaactgaaagggggttcaggcgggtcgggtggcgtgagcaagggcgaggagctgttcaccggggtggtgcccatcctggtcgagctggacggcgacgtaaacggccacaagttcagcgtgcgcggcgagggcgagggcgatgccaccaacggcaagctgaccctgaagttcatctgcaccaccggcaagctgcccgtgccctggcccaccctcgtgaccaccctgacctacggcgtgcagtgcttcagccgctaccccgaccacatgaagcgccacgacttcttcaagtccgccatgcccgaaggctacgtccaggagcgcaccatcagcttcaaggacgacggcacctacaagacccgcgccgaggtgaagttcgagggcgacaccctggtgaaccgcatcgagctgaagggcatcgacttcaaggaggacggcaacatcctggggcacaagctggagtacaacttcaacagccacaacgtctatatcaccgccgacaagcagaagaacggcatcaaggccaacttcaagatccgccacaacgtggaggacggcagcgtgcagctcgccgaccactaccagcagaacacccccatcggcgacggccccgtgctgctgcccgacaaccactacctgagcacccagtccgtgctgagcaaagaccccaacgagaagcgcgatcacatggtcctgctggagttcgtgaccgccgccgggatcactcacggcatggacgagctgtacaagggtgggggtgggagcggcggcggtggctccgcggccaacgatgaaaactattctgaaaactatgcggatgcgtcttaatgacgaatccatgtgggagtttattcttgacacagatatttatgatataataactgagtaagcttaacataaggaggaaaaacatatgttgcgtagctctaacgatgtgacgcaacaaggttcgcgtccaaagacaaaattgggaggcagtagcatggggatcattcgcacttgtcgcctggggccagaccaggtgaagtcaatgcgtgcggctctggacttattcgggcgcgaatttggagatgtagccacttactcacagcaccaaccggacagtgattacttggggaatttacttcgcagtaaaacttttatcgctttggccgctttcgaccaggaggctgtagtaggtgcgttggcagcctatgttcttcctaaattcgagcaaccgcgtagcgaaatttacatctatgatcttgcagtctccggcgaacatcgccgtcaggggatcgccacagctttaatcaaccttttgaagcatgaggctaatgcacttggagcgtacgtgatttatgtgcaggctgactacggtgatgatcctgcagtcgctctgtacaccaaactgggtatccgcgaggaggtcatgcactttgatattgacccgtcgacggctacctaagttctgttggtaaagatgggcggcgttctgccgcccgttatctctgttatacctttctgatatttgttatcgccgatccgtctttctccccttcccgccttgcgtcagg

SEQ ID NO: 23 - DNA, 19 bp, Artificial Sequence
  Synthetic
gcaaaatgctggctcattg

SEQ ID NO: 24 - DNA, 22 bp, Artificial Sequence
  Synthetic
gcgatgaatgtcttactacgga

SEQ ID NO: 25 - DNA, 20 bp, Artificial Sequence
  Synthetic
tatcatcctgaaagcgatgg

SEQ ID NO: 26 - DNA, 18 bp, Artificial Sequence
  Synthetic
actgaagcccagacgatc

SEQ ID NO: 27 - DNA, 17 bp, Artificial Sequence
  Synthetic
ctgctggaaaccatgcg

SEQ ID NO: 28 - DNA, 24 bp, Artificial Sequence
  Synthetic
caaaagagattctgggtattcact

SEQ ID NO: 29 - DNA, 21 bp, Artificial Sequence
  Synthetic
gagcatggtgatcttctcagt

SEQ ID NO: 30 - DNA, 17 bp, Artificial Sequence
  Synthetic
agatggcgagctggata

SEQ ID NO: 31 - DNA, 22 bp, Artificial Sequence
  Synthetic
agtactcaaccaagtcattctg